European Patent Specification EP 3 573 647 B1, published April 5, 2023. Title: Novel peptides and combination of peptides for use in immunotherapy against ovarian cancer and other cancers. Applicant: Immatics Biotechnologies GmbH. The sequence listing filed with the application follows.

SEQUENCE LISTING (776 sequences)

SEQ ID NO: 1 - protein, 9 aa, Homo sapiens
MIPTFTALL

SEQ ID NO: 2 - protein, 9 aa, Homo sapiens
TLLKALLEI

SEQ ID NO: 3 - protein, 9 aa, Homo sapiens
ALIYNLVGI

SEQ ID NO: 4 - protein, 8 aa, Homo sapiens
ALFKAWAL

SEQ ID NO: 5 - protein, 9 aa, Homo sapiens
RLLDFINVL

SEQ ID NO: 6 - protein, 9 aa, Homo sapiens
SLGKHTVAL

SEQ ID NO: 7 - protein, 9 aa, Homo sapiens
ALQAFEFRV

SEQ ID NO: 8 - protein, 9 aa, Homo sapiens
YLVTKVVAV

SEQ ID NO: 9 - protein, 10 aa, Homo sapiens
VLLAGFKPPL

SEQ ID NO: 10 - protein, 11 aa, Homo sapiens
RYSDSVGRVSF

SEQ ID NO: 11 - protein, 9 aa, Homo sapiens
SYSDLHYGF

SEQ ID NO: 12 - protein, 9 aa, Homo sapiens
KYEKIFEML

SEQ ID NO: 13 - protein, 9 aa, Homo sapiens
VYTFLSSTL

SEQ ID NO: 14 - protein, 9 aa, Homo sapiens
FYFPTPTVL

SEQ ID NO: 15 - protein, 10 aa, Homo sapiens
VYHDDKQPTF

SEQ ID NO: 16 - protein, 9 aa, Homo sapiens
IYSPQFSRL

SEQ ID NO: 17 - protein, 9 aa, Homo sapiens
RFTTMLSTF

SEQ ID NO: 18 - protein, 9 aa, Homo sapiens
KYPVHIYRL

SEQ ID NO: 19 - protein, 9 aa, Homo sapiens
KYVKVFHQF

SEQ ID NO: 20 - protein, 9 aa, Homo sapiens
RMASPVNVK

SEQ ID NO: 21 - protein, 9 aa, Homo sapiens
AVRKPIVLK

SEQ ID NO: 22 - protein, 9 aa, Homo sapiens
SLKERNPLK

SEQ ID NO: 23 - protein, 9 aa, Homo sapiens
GMMKGGIRK

SEQ ID NO: 24 - protein, 9 aa, Homo sapiens
SMYYPLQLK

SEQ ID NO: 25 - protein, 9 aa, Homo sapiens
GTSPPSVEK

SEQ ID NO: 26 - protein, 9 aa, Homo sapiens
RISEYLLEK

SEQ ID NO: 27 - protein, 10 aa, Homo sapiens
VLYGPAGLGK

SEQ ID NO: 28 - protein, 11 aa, Homo sapiens
KTYETNLEIKK

SEQ ID NO: 29 - protein, 9 aa, Homo sapiens
QQFLTALFY

SEQ ID NO: 30 - protein, 9 aa, Homo sapiens
ALEVAHRLK

SEQ ID NO: 31 - protein, 10 aa, Homo sapiens
LLDEGAMLLY

SEQ ID NO: 32 - protein, 9 aa, Homo sapiens
SPNKGTLSV

SEQ ID NO: 33 - protein, 8 aa, Homo sapiens
SPTFHLTL

SEQ ID NO: 34 - protein, 10 aa, Homo sapiens
LPRGPLASLL

SEQ ID NO: 35 - protein, 9 aa, Homo sapiens
FPDNQRPAL

SEQ ID NO: 36 - protein, 9 aa, Homo sapiens
APAAWLRSA

SEQ ID NO: 37 - protein, 9 aa, Homo sapiens
RPLFQKSSM

SEQ ID NO: 38 - protein, 11 aa, Homo sapiens
SPHPVTALLTL

SEQ ID NO: 39 - protein, 9 aa, Homo sapiens
RPAPFEVVF

SEQ ID NO: 40 - protein, 10 aa, Homo sapiens
KPGTSYRVTL

SEQ ID NO: 41 - protein, 9 aa, Homo sapiens
RVRSRISNL

SEQ ID NO: 42 - protein, 8 aa, Homo sapiens
TLKVTSAL

SEQ ID NO: 43 - protein, 9 aa, Homo sapiens
ALKARTVTF

SEQ ID NO: 44 - protein, 8 aa, Homo sapiens
LNKQKVTF

SEQ ID NO: 45 - protein, 9 aa, Homo sapiens
VGREKKLAL

SEQ ID NO: 46 - protein, 9 aa, Homo sapiens
DMKKAKEQL

SEQ ID NO: 47 - protein, 9 aa, Homo sapiens
MPNLRSVDL

SEQ ID NO: 48 - protein, 9 aa, Homo sapiens
DVKKKIKEV

SEQ ID NO: 49 - protein, 9 aa, Homo sapiens
LPRLKAFMI

SEQ ID NO: 50 - protein, 8 aa, Homo sapiens
DMKYKNRV

SEQ ID NO: 51 - protein, 9 aa, Homo sapiens
SLRLKNVQL

SEQ ID NO: 52 - protein, 9 aa, Homo sapiens
AEFLLRIFL

SEQ ID NO: 53 - protein, 9 aa, Homo sapiens
MEHPGKLLF

SEQ ID NO: 54 - protein, 11 aa, Homo sapiens
AEITITTQTGY

SEQ ID NO: 55 - protein, 9 aa, Homo sapiens
HETETRTTW

SEQ ID NO: 56 - protein, 9 aa, Homo sapiens
SEPDTTASW

SEQ ID NO: 57 - protein, 9 aa, Homo sapiens
QESDLRLFL

SEQ ID NO: 58 - protein, 8 aa, Homo sapiens
GEMEQKQL

SEQ ID NO: 59 - protein, 9 aa, Homo sapiens
SENVTMKVV

SEQ ID NO: 60 - protein, 11 aa, Homo sapiens
GLLSLTSTLYL

SEQ ID NO: 61 - protein, 9 aa, Homo sapiens
YMVHIQVTL

SEQ ID NO: 62 - protein, 9 aa, Homo sapiens
KVLGVNVML

SEQ ID NO: 63 - protein, 9 aa, Homo sapiens
MMEEMIFNL

SEQ ID NO: 64 - protein, 9 aa, Homo sapiens
FLDPDRHFL

SEQ ID NO: 65 - protein, 9 aa, Homo sapiens
TMFLRETSL

SEQ ID NO: 66 - protein, 9 aa, Homo sapiens
GLLQELSSI

SEQ ID NO: 67 - protein, 9 aa, Homo sapiens
SLLLPSIFL

SEQ ID NO: 68 - protein, 9 aa, Homo sapiens
KLFDTQQFL

SEQ ID NO: 69 - protein, 9 aa, Homo sapiens
TTYEGSITV

SEQ ID NO: 70 - protein, 9 aa, Homo sapiens
VLQGLLRSL

SEQ ID NO: 71 - protein, 9 aa, Homo sapiens
YLEDTDRNL

SEQ ID NO: 72 - protein, 9 aa, Homo sapiens
YLTDLQVSL

SEQ ID NO: 73 - protein, 9 aa, Homo sapiens
FLIEELLFA

SEQ ID NO: 74 - protein, 9 aa, Homo sapiens
SQSPSVSQL

SEQ ID NO: 75 - protein, 9 aa, Homo sapiens
KVVSVLYNV

SEQ ID NO: 76 - protein, 9 aa, Homo sapiens
KYVAELSLL

SEQ ID NO: 77 - protein, 8 aa, Homo sapiens
RYGPVFTV

SEQ ID NO: 78 - protein, 9 aa, Homo sapiens
SFAPRSAVF

SEQ ID NO: 79 - protein, 9 aa, Homo sapiens
SYNEHWNYL

SEQ ID NO: 80 - protein, 10 aa, Homo sapiens
TAYMVSVAAF

SEQ ID NO: 81 - protein, 9 aa, Homo sapiens
VYNHTTRPL

SEQ ID NO: 82 - protein, 9 aa, Homo sapiens
SYFRGFTLI

SEQ ID NO: 83 - protein, 9 aa, Homo sapiens
GTYAHTVNR

SEQ ID NO: 84 - protein, 10 aa, Homo sapiens
KLQPAQTAAK

SEQ ID NO: 85 - protein, 10 aa, Homo sapiens
VLLGSLFSRK

SEQ ID NO: 86 - protein, 11 aa, Homo sapiens
VVLLGSLFSRK

SEQ ID NO: 87 - protein, 10 aa, Homo sapiens
AVAPPTPASK

SEQ ID NO: 88 - protein, 9 aa, Homo sapiens
VVHAVFALK

SEQ ID NO: 89 - protein, 9 aa, Homo sapiens
RVAELLLLH

SEQ ID NO: 90 - protein, 10 aa, Homo sapiens
KVAGERYVYK

SEQ ID NO: 91 - protein, 9 aa, Homo sapiens
RSLRYYYEK

SEQ ID NO: 92 - protein, 9 aa, Homo sapiens
SVFPIENIY

SEQ ID NO: 93 - protein, 9 aa, Homo sapiens
KILEEHTNK

SEQ ID NO: 94 - protein, 9 aa, Homo sapiens
ATFERVLLR

SEQ ID NO: 95 - protein, 10 aa, Homo sapiens
QSMYYPLQLK

SEQ ID NO: 96 - protein, 9 aa, Homo sapiens
TAFGGFLKY

SEQ ID NO: 97 - protein, 10 aa, Homo sapiens
TMLDVEGLFY

SEQ ID NO: 98 - protein, 10 aa, Homo sapiens
LLQPPPLLAR

SEQ ID NO: 99 - protein, 9 aa, Homo sapiens
KVVDRWNEK

SEQ ID NO: 100 - protein, 10 aa, Homo sapiens
RLFTSPIMTK

SEQ ID NO: 101 - protein, 10 aa, Homo sapiens
RVFTSSIKTK

SEQ ID NO: 102 - protein, 9 aa, Homo sapiens
SVLTSSLVK

SEQ ID NO: 103 - protein, 9 aa, Homo sapiens
TSRSVDEAY

SEQ ID NO: 104 - protein, 9 aa, Homo sapiens
VLADSVTTK

SEQ ID NO: 105 - protein, 9 aa, Homo sapiens
RLFSWLVNR

SEQ ID NO: 106 - protein, 9 aa, Homo sapiens
AAFVPLLLK

SEQ ID NO: 107 - protein, 9 aa, Homo sapiens
RLQEWKALK

SEQ ID NO: 108 - protein, 10 aa, Homo sapiens
VLYPVPLESY

SEQ ID NO: 109 - protein, 11 aa, Homo sapiens
KTFTIKRFLAK

SEQ ID NO: 110 - protein, 9 aa, Homo sapiens
SAAPPSYFR

SEQ ID NO: 111 - protein, 10 aa, Homo sapiens
TLPQFRELGY

SEQ ID NO: 112 - protein, 10 aa, Homo sapiens
TVTGAEQIQY

SEQ ID NO: 113 - protein, 9 aa, Homo sapiens
QLDSNRLTY

SEQ ID NO: 114 - protein, 10 aa, Homo sapiens
VMEQSAGIMY

SEQ ID NO: 115 - protein, 9 aa, Homo sapiens
FVDNQYWRY

SEQ ID NO: 116 - protein, 11 aa, Homo sapiens
VLLDEGAMLLY

SEQ ID NO: 117 - protein, 10 aa, Homo sapiens
APRLLLLAVL

SEQ ID NO: 118 - protein, 9 aa, Homo sapiens
SPASRSISL

SEQ ID NO: 119 - protein, 10 aa, Homo sapiens
APLPRPGAVL

SEQ ID NO: 120 - protein, 9 aa, Homo sapiens
RPAMNYDKL

SEQ ID NO: 121 - protein, 9 aa, Homo sapiens
VPNQSSESL

SEQ ID NO: 122 - protein, 9 aa, Homo sapiens
YPGFPQSQY

SEQ ID NO: 123 - protein, 10 aa, Homo sapiens
KPSESIYSAL

SEQ ID NO: 124 - protein, 11 aa, Homo sapiens
LPSDSHFKITF

SEQ ID NO: 125 - protein, 10 aa, Homo sapiens
VPVYILLDEM

SEQ ID NO: 126 - protein, 8 aa, Homo sapiens
KPGPEDKL

SEQ ID NO: 127 - protein, 9 aa, Homo sapiens
APRAGSQVV

SEQ ID NO: 128 - protein, 9 aa, Homo sapiens
YPRTITPGM

SEQ ID NO: 129 - protein, 8 aa, Homo sapiens
APRPASSL

SEQ ID NO: 130 - protein, 9 aa, Homo sapiens
FPRLVGPDF

SEQ ID NO: 131 - protein, 9 aa, Homo sapiens
APTEDLKAL

SEQ ID NO: 132 - protein, 9 aa, Homo sapiens
IPGPAQSTI

SEQ ID NO: 133 - protein, 10 aa, Homo sapiens
MPNLPSTTSL

SEQ ID NO: 134 - protein, 9 aa, Homo sapiens
RPIVPGPLL

SEQ ID NO: 135 - protein, 9 aa, Homo sapiens
RVRSTISSL

SEQ ID NO: 136 - protein, 11 aa, Homo sapiens
SPFSAEEANSL

SEQ ID NO: 137 - protein, 10 aa, Homo sapiens
SPGATSRGTL

SEQ ID NO: 138 - protein, 9 aa, Homo sapiens
SPMATTSTL

SEQ ID NO: 139 - protein, 9 aa, Homo sapiens
SPQSMSNTL

SEQ ID NO: 140 - protein, 11 aa, Homo sapiens
SPRTEASSAVL

SEQ ID NO: 141 - protein, 11 aa, Homo sapiens
SPMTSLLTSGL

SEQ ID NO: 142 - protein, 9 aa, Homo sapiens
TPGLRETSI

SEQ ID NO: 143 - protein, 9 aa, Homo sapiens
SPAMTSTSF

SEQ ID NO: 144 - protein, 9 aa, Homo sapiens
SPSPVSSTL

SEQ ID NO: 145 - protein, 9 aa, Homo sapiens
SPSSPMSTF

SEQ ID NO: 146 - protein, 9 aa, Homo sapiens
IPRPEVQAL

SEQ ID NO: 147 - protein, 11 aa, Homo sapiens
APRWFPQPTVV

SEQ ID NO: 148 - protein, 9 aa, Homo sapiens
KPYGGSGPL

SEQ ID NO: 149 - protein, 9 aa, Homo sapiens
GPREALSRL

SEQ ID NO: 150 - protein, 8 aa, Homo sapiens
MAAVKQAL

SEQ ID NO: 151 - protein, 9 aa, Homo sapiens
HLLLKVLAF

SEQ ID NO: 152 - protein, 9 aa, Homo sapiens
MGSARVAEL

SEQ ID NO: 153 - protein, 9 aa, Homo sapiens
NAMLRKVAV

SEQ ID NO: 154 - protein, 9 aa, Homo sapiens
MLRKIAVAA

SEQ ID NO: 155 - protein, 9 aa, Homo sapiens
NKKMMKRLM

SEQ ID NO: 156 - protein, 8 aa, Homo sapiens
HVKEKFLL

SEQ ID NO: 157 - protein, 9 aa, Homo sapiens
EAMKRLSYI

SEQ ID NO: 158 - protein, 8 aa, Homo sapiens
LPKLAGLL

SEQ ID NO: 159 - protein, 9 aa, Homo sapiens
VLKHKLDEL

SEQ ID NO: 160 - protein, 8 aa, Homo sapiens
YPKARLAF

SEQ ID NO: 161 - protein, 9 aa, Homo sapiens
ALKTTTTAL

SEQ ID NO: 162 - protein, 8 aa, Homo sapiens
QAKTHSTL

SEQ ID NO: 163 - protein, 8 aa, Homo sapiens
QGLLRPVF

SEQ ID NO: 164 - protein, 9 aa, Homo sapiens
SIKTKSAEM

SEQ ID NO: 165 - protein, 8 aa, Homo sapiens
SPRFKTGL

SEQ ID NO: 166 - protein, 9 aa, Homo sapiens
TPKLRETSI

SEQ ID NO: 167 - protein, 9 aa, Homo sapiens
TSHERLTTL

SEQ ID NO: 168 - protein, 9 aa, Homo sapiens
TSHERLTTY

SEQ ID NO: 169 - protein, 9 aa, Homo sapiens
TSMPRSSAM

SEQ ID NO: 170 - protein, 9 aa, Homo sapiens
YLLEKSRVI

SEQ ID NO: 171 - protein, 8 aa, Homo sapiens
FAFRKEAL

SEQ ID NO: 172 - protein, 9 aa, Homo sapiens
KLKERNREL

SEQ ID NO: 173 - protein, 11 aa, Homo sapiens
AEAQVGDERDY

SEQ ID NO: 174 - protein, 10 aa, Homo sapiens
AEATARLNVF

SEQ ID NO: 175 - protein, 9 aa, Homo sapiens
AEIEPKADG

SEQ ID NO: 176 - protein, 11 aa, Homo sapiens
AEIEPKADGSW

SEQ ID NO: 177 - protein, 9 aa, Homo sapiens
TEVGTMNLF

SEQ ID NO: 178 - protein, 10 aa, Homo sapiens
NELFRDGVNW

SEQ ID NO: 179 - protein, 9 aa, Homo sapiens
REAGDEFEL

SEQ ID NO: 180 - protein, 11 aa, Homo sapiens
REAGDEFELRY

SEQ ID NO: 181 - protein, 8 aa, Homo sapiens
GEGPKTSW

SEQ ID NO: 182 - protein, 9 aa, Homo sapiens
KEATEAQSL

SEQ ID NO: 183 - protein, 9 aa, Homo sapiens
YEKGIMQKV

SEQ ID NO: 184 - protein, 10 aa, Homo sapiens
AELEALTDLW

SEQ ID NO: 185 - protein, 10 aa, Homo sapiens
AERQPGAASL

SEQ ID NO: 186 - protein, 9 aa, Homo sapiens
REGPEEPGL

SEQ ID NO: 187 - protein, 9 aa, Homo sapiens
GEAQTRIAW

SEQ ID NO: 188 - protein, 10 aa, Homo sapiens
AEFAKKQPWW

SEQ ID NO: 189 - protein, 8 aa, Homo sapiens
KEFLFNMY

SEQ ID NO: 190 - protein, 9 aa, Homo sapiens
YEVARILNL

SEQ ID NO: 191 - protein, 10 aa, Homo sapiens
EEDAALFKAW

SEQ ID NO: 192 - protein, 9 aa, Homo sapiens
YEFKFPNRL

SEQ ID NO: 193 - protein, 8 aa, Homo sapiens
LEAQQEAL

SEQ ID NO: 194 - protein, 10 aa, Homo sapiens
KEVDPTSHSY

SEQ ID NO: 195 - protein, 9 aa, Homo sapiens
AEDKRHYSV

SEQ ID NO: 196 - protein, 9 aa, Homo sapiens
REMPGGPVW

SEQ ID NO: 197 - protein, 9 aa, Homo sapiens
AEVLLPRLV

SEQ ID NO: 198 - protein, 8 aa, Homo sapiens
QEAARAAL

SEQ ID NO: 199 - protein, 10 aa, Homo sapiens
REIDESLIFY

SEQ ID NO: 200 - protein, 9 aa, Homo sapiens
AESIPTVSF

SEQ ID NO: 201 - protein, 10 aa, Homo sapiens
AETILTFHAF

SEQ ID NO: 202 - protein, 9 aa, Homo sapiens
HESEATASW

SEQ ID NO: 203 - protein, 11 aa, Homo sapiens
IEHSTQAQDTL

SEQ ID NO: 204 - protein, 11 aa, Homo sapiens
RETSTSEETSL

SEQ ID NO: 205 - protein, 8 aa, Homo sapiens
SEITRIEM

SEQ ID NO: 206 - protein, 10 aa, Homo sapiens
SESVTSRTSY

SEQ ID NO: 207 - protein, 10 aa, Homo sapiens
TEARATSDSW

SEQ ID NO: 208 - protein, 9 aa, Homo sapiens
TEVSRTEAI

SEQ ID NO: 209 - protein, 8 aa, Homo sapiens
TEVSRTEL

SEQ ID NO: 210 - protein, 10 aa, Homo sapiens
VEAADIFQNF

SEQ ID NO: 211 - protein, 10 aa, Homo sapiens
EEKVFPSPLW

SEQ ID NO: 212 - protein, 10 aa, Homo sapiens
MEQKQLQKRF

SEQ ID NO: 213 - protein, 9 aa, Homo sapiens
KESIPRWYY

SEQ ID NO: 214 - protein, 10 aa, Homo sapiens
VEQTRAGSLL

SEQ ID NO: 215 - protein, 11 aa, Homo sapiens
SEDGLPEGIHL

SEQ ID NO: 216 - protein, 10 aa, Homo sapiens
IMFDDAIERA

SEQ ID NO: 217 - protein, 9 aa, Homo sapiens
VSSSLTLKV

SEQ ID NO: 218 - protein, 10 aa, Homo sapiens
TIASQRLTPL

SEQ ID NO: 219 - protein, 9 aa, Homo sapiens
PLPRPGAVL

SEQ ID NO: 220 - protein, 9 aa, Homo sapiens
RMTTQLLLL

SEQ ID NO: 221 - protein, 8 aa, Homo sapiens
SLLDLYQL

SEQ ID NO: 222 - protein, 10 aa, Homo sapiens
ALMRLIGCPL

SEQ ID NO: 223 - protein, 8 aa, Homo sapiens
FAHHGRSL

SEQ ID NO: 224 - protein, 9 aa, Homo sapiens
SLPRFQVTL

SEQ ID NO: 225 - protein, 9 aa, Homo sapiens
SVFAHPRKL

SEQ ID NO: 226 - protein, 10 aa, Homo sapiens
QVDPKKRISM

SEQ ID NO: 227 - protein, 9 aa, Homo sapiens
YTFRYPLSL

SEQ ID NO: 228 - protein, 9 aa, Homo sapiens
RLWDWVPLA

SEQ ID NO: 229 - protein, 9 aa, Homo sapiens
ISVPAKTSL

SEQ ID NO: 230 - protein, 9 aa, Homo sapiens
SAFREGTSL

SEQ ID NO: 231 - protein, 9 aa, Homo sapiens
SVTESTHHL

SEQ ID NO: 232 - protein, 9 aa, Homo sapiens
TISSLTHEL

SEQ ID NO: 233 - protein, 9 aa, Homo sapiens
GSDTSSKSL

SEQ ID NO: 234 - protein, 9 aa, Homo sapiens
GVATRVDAI

SEQ ID NO: 235 - protein, 9 aa, Homo sapiens
SAIETSAVL

SEQ ID NO: 236 - protein, 9 aa, Homo sapiens
SAIPFSMTL

SEQ ID NO: 237 - protein, 9 aa, Homo sapiens
SAMGTISIM

SEQ ID NO: 238 - protein, 8 aa, Homo sapiens
PLLVLFTI

SEQ ID NO: 239 - protein, 9 aa, Homo sapiens
FAVPTGISM

SEQ ID NO: 240 - protein, 9 aa, Homo sapiens
FSTDTSIVL

SEQ ID NO: 241 - protein, 9 aa, Homo sapiens
RQPNILVHL

SEQ ID NO: 242 - protein, 9 aa, Homo sapiens
STIPALHEI

SEQ ID NO: 243 - protein, 9 aa, Homo sapiens
YASEGVKQV

SEQ ID NO: 244 - protein, 10 aa, Homo sapiens
DTDSSVHVQV

SEQ ID NO: 245 - protein, 9 aa, Homo sapiens
LAVEGGQSL

SEQ ID NO: 246 - protein, 10 aa, Homo sapiens
RYLAVVHAVF

SEQ ID NO: 247 - protein, 9 aa, Homo sapiens
ARPPWMWVL

SEQ ID NO: 248 - protein, 8 aa, Homo sapiens
SVIQHLGY

SEQ ID NO: 249 - protein, 9 aa, Homo sapiens
VYTPTLGTL

SEQ ID NO: 250 - protein, 10 aa, Homo sapiens
HFPEKTTHSF

SEQ ID NO: 251 - protein, 9 aa, Homo sapiens
KQRQVLIFF

SEQ ID NO: 252 - protein, 9 aa, Homo sapiens
LYQPRASEM

SEQ ID NO: 253 - protein, 8 aa, Homo sapiens
AYPEIEKF

SEQ ID NO: 254 - protein, 9 aa, Homo sapiens
IIQHLTEQF

SEQ ID NO: 255 - protein, 9 aa, Homo sapiens
VFVSFSSLF

SEQ ID NO: 256 - protein, 10 aa, Homo sapiens
RTEEVLLTFK

SEQ ID NO: 257 - protein, 9 aa, Homo sapiens
VTADHSHVF

SEQ ID NO: 258 - protein, 9 aa, Homo sapiens
GAYAHTVNR

SEQ ID NO: 259 - protein, 9 aa, Homo sapiens
KTLELRVAY

SEQ ID NO: 260 - protein, 9 aa, Homo sapiens
GTNTVILEY

SEQ ID NO: 261 - protein, 9 aa, Homo sapiens
HTFGLFYQR

SEQ ID NO: 262 - protein, 10 aa, Homo sapiens
RSRLNPLVQR

SEQ ID NO: 263 - protein, 9 aa, Homo sapiens
SSSSATISK

SEQ ID NO: 264 - protein, 10 aa, Homo sapiens
AIKVIPTVFK

SEQ ID NO: 265 - protein, 9 aa, Homo sapiens
QIHDHVNPK

SEQ ID NO: 266 - protein, 10 aa, Homo sapiens
ISYSGQFLVK

SEQ ID NO: 267 - protein, 9 aa, Homo sapiens
VTDLISPRK

SEQ ID NO: 268 - protein, 9 aa, Homo sapiens
GLLGLSLRY

SEQ ID NO: 269 - protein, 10 aa, Homo sapiens
RLKGDAWVYK

SEQ ID NO: 270 - protein, 11 aa, Homo sapiens
AVFNPRFYRTY

SEQ ID NO: 271 - protein, 12 aa, Homo sapiens
RMFADDLHNLNK

SEQ ID NO: 272 - protein, 11 aa, Homo sapiens
RQPERTILRPR

SEQ ID NO: 273 - protein, 9 aa, Homo sapiens
RVNAIPFTY

SEQ ID NO: 274 - protein, 9 aa, Homo sapiens
KTFPASTVF

SEQ ID NO: 275 - protein, 9 aa, Homo sapiens
STTFPTLTK

SEQ ID NO: 276 - protein, 9 aa, Homo sapiens
VSKTTGMEF

SEQ ID NO: 277 - protein, 9 aa, Homo sapiens
TTALKTTSR

SEQ ID NO: 278 - protein, 9 aa, Homo sapiens
NLSSITHER

SEQ ID NO: 279 - protein, 11 aa, Homo sapiens
SVSSETTKIKR

SEQ ID NO: 280 - protein, 9 aa, Homo sapiens
SVSGVKTTF

SEQ ID NO: 281 - protein, 9 aa, Homo sapiens
RAKELEATF

SEQ ID NO: 282 - protein, 11 aa, Homo sapiens
CLTRTGLFLRF

SEQ ID NO: 283 - protein, 9 aa, Homo sapiens
IVQEPTEEK

SEQ ID NO: 284 - protein, 9 aa, Homo sapiens
KSLIKSWKK

SEQ ID NO: 285 - protein, 9 aa, Homo sapiens
GTVNPTVGK

SEQ ID NO: 286 - protein, 10 aa, Homo sapiens
TVAPPQGVVK

SEQ ID NO: 287 - protein, 11 aa, Homo sapiens
RRIHTGEKPYK

SEQ ID NO: 288 - protein, 11 aa, Homo sapiens
SPVTSVHGGTY

SEQ ID NO: 289 - protein, 9 aa, Homo sapiens
RWEKTDLTY

SEQ ID NO: 290 - protein, 10 aa, Homo sapiens
DMDEEIEAEY

SEQ ID NO: 291 - protein, 9 aa, Homo sapiens
ETIRSVGYY

SEQ ID NO: 292 - protein, 11 aa, Homo sapiens
NVTMKVVSVLY

SEQ ID NO: 293 - protein, 11 aa, Homo sapiens
VPDSGATATAY

SEQ ID NO: 294 - protein, 9 aa, Homo sapiens
YPLRGSSIF

SEQ ID NO: 295 - protein, 11 aa, Homo sapiens
YPLRGSSIFGL

SEQ ID NO: 296 - protein, 8 aa, Homo sapiens
YPLRGSSI

SEQ ID NO: 297 - protein, 9 aa, Homo sapiens
TVREASGLL

SEQ ID NO: 298 - protein, 8 aa, Homo sapiens
YPTEHVQF

SEQ ID NO: 299 - protein, 9 aa, Homo sapiens
HPGSSALHY

SEQ ID NO: 300 - protein, 10 aa, Homo sapiens
IPMAAVKQAL

SEQ ID NO: 301 - protein, 10 aa, Homo sapiens
SPRRSPRISF

SEQ ID NO: 302 - protein, 9 aa, Homo sapiens
RVEEVRALL

SEQ ID NO: 303 - protein, 9 aa, Homo sapiens
LPMWKVTAF

SEQ ID NO: 304 - protein, 8 aa, Homo sapiens
LPRPGAVL

SEQ ID NO: 305 - protein, 10 aa, Homo sapiens
TPWAESSTKF

SEQ ID NO: 306 - protein, 9 aa, Homo sapiens
APVIFSHSA

SEQ ID NO: 307 - protein, 12 aa, Homo sapiens
LPYGPGSEAAAF

SEQ ID NO: 308 - protein, 9 aa, Homo sapiens
YPEGAAYEF

SEQ ID NO: 309 - protein, 9 aa, Homo sapiens
FPQSQYPQY

SEQ ID NO: 310 - protein, 9 aa, Homo sapiens
RPNPITIIL

SEQ ID NO: 311 - protein, 9 aa, Homo sapiens
RPLFYVVSL

SEQ ID NO: 312 - protein, 9 aa, Homo sapiens
LPYFREFSM

SEQ ID NO: 313 - protein, 9 aa, Homo sapiens
KVKSDRSVF

SEQ ID NO: 314 - protein, 9 aa, Homo sapiens
VPDQPHPEI

SEQ ID NO: 315 - protein, 10 aa, Homo sapiens
SPRENFPDTL

SEQ ID NO: 316 - protein, 8 aa, Homo sapiens
EPKTATVL

SEQ ID NO: 317 - protein, 8 aa, Homo sapiens
FPFQPGSV

SEQ ID NO: 318 - protein, 9 aa, Homo sapiens
FPNRLNLEA

SEQ ID NO: 319 - protein, 11 aa, Homo sapiens
SPAEPSVYATL

SEQ ID NO: 320 - protein, 9 aa, Homo sapiens
FPMSPVTSV

SEQ ID NO: 321 - protein, 9 aa, Homo sapiens
SPMDTFLLI

SEQ ID NO: 322 - protein, 9 aa, Homo sapiens
SPDPSKHLL

SEQ ID NO: 323 - protein, 9 aa, Homo sapiens
RPMPNLRSV

SEQ ID NO: 324 - protein, 8 aa, Homo sapiens
VPYRVVGL

SEQ ID NO: 325 - protein, 9 aa, Homo sapiens
GPRNAQRVL

SEQ ID NO: 326 - protein, 9 aa, Homo sapiens
VPSEIDAAF

SEQ ID NO: 327 - protein, 9 aa, Homo sapiens
SPLPVTSLI

SEQ ID NO: 328 - protein, 10 aa, Homo sapiens
EPVTSSLPNF

SEQ ID NO: 329 - protein, 12 aa, Homo sapiens
FPAMTESGGMIL

SEQ ID NO: 330 - protein, 10 aa, Homo sapiens
FPFVTGSTEM

SEQ ID NO: 331 - protein, 10 aa, Homo sapiens
FPHPEMTTSM

SEQ ID NO: 332 - protein, 9 aa, Homo sapiens
FPHSEMTTL

SEQ ID NO: 333 - protein, 10 aa, Homo sapiens
FPHSEMTTVM

SEQ ID NO: 334 - protein, 9 aa, Homo sapiens
FPYSEVTTL

SEQ ID NO: 335 - protein, 9 aa, Homo sapiens
HPDPVGPGL

SEQ ID NO: 336 - protein, 12 aa, Homo sapiens
HPKTESATPAAY

SEQ ID NO: 337 - protein, 9 aa, Homo sapiens
HPVETSSAL

SEQ ID NO: 338 - protein, 9 aa, Homo sapiens
HVTKTQATF

SEQ ID NO: 339 - protein, 11 aa, Homo sapiens
LPAGTTGSLVF

SEQ ID NO: 340 - protein, 9 aa, Homo sapiens
LPEISTRTM

SEQ ID NO: 341 - protein, 9 aa, Homo sapiens
LPLDTSTTL

SEQ ID NO: 342 - protein, 9 aa, Homo sapiens
LPLGTSMTF

SEQ ID NO: 343 - protein, 11 aa, Homo sapiens
LPSVSGVKTTF

SEQ ID NO: 344 - protein, 9 aa, Homo sapiens
LPTQTTSSL

SEQ ID NO: 345 - protein, 10 aa, Homo sapiens
LPTSESLVSF

SEQ ID NO: 346 - protein, 10 aa, Homo sapiens
LPWDTSTTLF

SEQ ID NO: 347 - protein, 10 aa, Homo sapiens
MPLTTGSQGM

SEQ ID NO: 348 - protein, 10 aa, Homo sapiens
MPNSAIPFSM

SEQ ID NO: 349 - protein, 11 aa, Homo sapiens
MPSLSEAMTSF

SEQ ID NO: 350 - protein, 9 aa, Homo sapiens
NPSSTTTEF

SEQ ID NO: 351 - protein, 9 aa, Homo sapiens
NVLTSTPAF

SEQ ID NO: 352 - protein, 9 aa, Homo sapiens
SPAETSTNM

SEQ ID NO: 353 - protein, 9 aa, Homo sapiens
SPAMTTPSL

SEQ ID NO: 354 - protein, 9 aa, Homo sapiens
SPLPVTSLL

SEQ ID NO: 355 - protein, 9 aa, Homo sapiens
SPLVTSHIM

SEQ ID NO: 356 - protein, 9 aa, Homo sapiens
SPNEFYFTV

SEQ ID NO: 357 - protein, 9 aa, Homo sapiens
SPSPVPTTL

SEQ ID NO: 358 - protein, 9 aa, Homo sapiens
SPSPVTSTL

SEQ ID NO: 359 - protein, 9 aa, Homo sapiens
SPSTIKLTM

SEQ ID NO: 360 - protein, 9 aa, Homo sapiens
SPSVSSNTY

SEQ ID NO: 361 - protein, 9 aa, Homo sapiens
SPTHVTQSL

SEQ ID NO: 362 - protein, 9 aa, Homo sapiens
SPVPVTSLF

SEQ ID NO: 363 - protein, 9 aa, Homo sapiens
TAKTPDATF

SEQ ID NO: 364 - protein, 9 aa, Homo sapiens
TPLATTQRF

SEQ ID NO: 365 - protein, 11 aa, Homo sapiens
TPLATTQRFTY

SEQ ID NO: 366 - protein, 11 aa, Homo sapiens
TPLTTTGSAEM

SEQ ID NO: 367 - protein, 9 aa, Homo sapiens
TPSVVTEGF

SEQ ID NO: 368 - protein, 9 aa, Homo sapiens
VPTPVFPTM

SEQ ID NO: 369 - protein, 9 aa, Homo sapiens
FPHSEMTTV

SEQ ID NO: 370 - protein, 8 aa, Homo sapiens
PGGTRQSL

SEQ ID NO: 371 - protein, 9 aa, Homo sapiens
LYVDGFTHW

SEQ ID NO: 372 - protein, 10 aa, Homo sapiens
IPRNPPPTLL

SEQ ID NO: 373 - protein, 11 aa, Homo sapiens
RPRALRDLRIL

SEQ ID NO: 374 - protein, 10 aa, Homo sapiens
NPIGDTGVKF

SEQ ID NO: 375 - protein, 9 aa, Homo sapiens
AAASPLLLL

SEQ ID NO: 376 - protein, 10 aa, Homo sapiens
RPRSPAGQVA

SEQ ID NO: 377 - protein, 12 aa, Homo sapiens
RPRSPAGQVAAA

SEQ ID NO: 378 - protein, 11 aa, Homo sapiens
RPRSPAGQVAA

SEQ ID NO: 379 - protein, 9 aa, Homo sapiens
GPFPLVYVL

SEQ ID NO: 380 - protein, 8 aa, Homo sapiens
IPTYGRTF

SEQ ID NO: 381 - protein, 9 aa, Homo sapiens
LPEQTPLAF

SEQ ID NO: 382 - protein, 9 aa, Homo sapiens
SPMHDRWTF

SEQ ID NO: 383 - protein, 9 aa, Homo sapiens
TPTKETVSL

SEQ ID NO: 384 - protein, 9 aa, Homo sapiens
YPGLRGSPM

SEQ ID NO: 385 - protein, 9 aa, Homo sapiens
SPALHIGSV

SEQ ID NO: 386 - protein, 8 aa, Homo sapiens
FPFNPLDF

SEQ ID NO: 387 - protein, 10 aa, Homo sapiens
APLKLSRTPA

SEQ ID NO: 388 - protein, 12 aa, Homo sapiens
SPAPLKLSRTPA

SEQ ID NO: 389 - protein, 11 aa, Homo sapiens
SPGAQRTFFQL

SEQ ID NO: 390 - protein, 9 aa, Homo sapiens
NPDLRRNVL

SEQ ID NO: 391 - protein, 10 aa, Homo sapiens
APSTPRITTF

SEQ ID NO: 392 - protein, 9 aa, Homo sapiens
KPIESTLVA

SEQ ID NO: 393 - protein, 8 aa, Homo sapiens
ASKPHVEI

SEQ ID NO: 394 - protein, 8 aa, Homo sapiens
MYKMKKPI

SEQ ID NO: 395 - protein, 9 aa, Homo sapiens
VLLPRLVSC

SEQ ID NO: 396 - protein, 9 aa, Homo sapiens
REASGLLSL

SEQ ID NO: 397 - protein, 9 aa, Homo sapiens
REGDTVQLL

SEQ ID NO: 398 - protein, 10 aa, Homo sapiens
SFEQVVNELF

SEQ ID NO: 399 - protein, 9 aa, Homo sapiens
RELLHLVTL

SEQ ID NO: 400 - protein, 8 aa, Homo sapiens
GEIEIHLL

SEQ ID NO: 401 - protein, 9 aa, Homo sapiens
EDLKEELLL

SEQ ID NO: 402 - protein, 10 aa, Homo sapiens
RELANDELIL

SEQ ID NO: 403 - protein, 9 aa, Homo sapiens
EEAQWVRKY

SEQ ID NO: 404 - protein, 8 aa, Homo sapiens
NEAIMHQY

SEQ ID NO: 405 - protein, 8 aa, Homo sapiens
NEIWTHSY

SEQ ID NO: 406 - protein, 9 aa, Homo sapiens
EDGRLVIEF

SEQ ID NO: 407 - protein, 9 aa, Homo sapiens
AEHEGVSVL

SEQ ID NO: 408 - protein, 8 aa, Homo sapiens
LEKALQVF

SEQ ID NO: 409 - protein, 12 aa, Homo sapiens
REFVLSKGDAGL

SEQ ID NO: 410 - protein, 9 aa, Homo sapiens
SEDPSKLEA

SEQ ID NO: 411 - protein, 9 aa, Homo sapiens
LELPPILVY

SEQ ID NO: 412 - protein, 9 aa, Homo sapiens
QEILTQVKQ

SEQ ID NO: 413 - protein, 10 aa, Homo sapiens
IEALSGKIEL

SEQ ID NO: 414 - protein, 9 aa, Homo sapiens
EDAALFKAW

SEQ ID NO: 415 - protein, 11 aa, Homo sapiens
REEDAALFKAW

SEQ ID NO: 416 - protein, 9 aa, Homo sapiens
SEEETRVVF

SEQ ID NO: 417 - protein, 9 aa, Homo sapiens
AEHFSMIRA

SEQ ID NO: 418 - protein, 9 aa, Homo sapiens
FEDAQGHIW

SEQ ID NO: 419 - protein, 9 aa, Homo sapiens
HEFGHVLGL

SEQ ID NO: 420 - protein, 9 aa, Homo sapiens
FESHSTVSA

SEQ ID NO: 421 - protein, 9 aa, Homo sapiens
GEPATTVSL

SEQ ID NO: 422 - protein, 9 aa, Homo sapiens
SETTFSLIF

SEQ ID NO: 423 - protein, 9 aa, Homo sapiens
SEVPTGTTA

SEQ ID NO: 424 - protein, 9 aa, Homo sapiens
TEFPLFSAA

SEQ ID NO: 425 - protein, 9 aa, Homo sapiens
SEVPLPMAI

SEQ ID NO: 426 - protein, 8 aa, Homo sapiens
PEKTTHSF

SEQ ID NO: 427 - protein, 9 aa, Homo sapiens
HESSSHHDL

SEQ ID NO: 428 - protein, 8 aa, Homo sapiens
LDLGLNHI

SEQ ID NO: 429 - protein, 9 aa, Homo sapiens
REKFIASVI

SEQ ID NO: 430 - protein, 9 aa, Homo sapiens
DEKILYPEF

SEQ ID NO: 431 - protein, 11 aa, Homo sapiens
AEQDPDELNKA

SEQ ID NO: 432 - protein, 8 aa, Homo sapiens
EEQYIAQF

SEQ ID NO: 433 - protein, 8 aa, Homo sapiens
SDSQVRAF

SEQ ID NO: 434 - protein, 9 aa, Homo sapiens
KEAIREHQM

SEQ ID NO: 435 - protein, 10 aa, Homo sapiens
REEFVSIDHL

SEQ ID NO: 436 - protein, 10 aa, Homo sapiens
REPGDIFSEL

SEQ ID NO: 437 - protein, 9 aa, Homo sapiens
TEAVVTNEL

SEQ ID NO: 438 - protein, 9 aa, Homo sapiens
SEVDSPNVL

SEQ ID NO: 439 - protein, 9 aa, Homo sapiens
EALAKLMSL

SEQ ID NO: 440 - protein, 9 aa, Homo sapiens
ELFEGLKAF

SEQ ID NO: 441 - protein, 9 aa, Homo sapiens
HQITEVGTM

SEQ ID NO: 442 - protein, 10 aa, Homo sapiens
ILSKLTDIQY

SEQ ID NO: 443 - protein, 9 aa, Homo sapiens
GTFNPVSLW

SEQ ID NO: 444 - protein, 9 aa, Homo sapiens
KLSQKGYSW

SEQ ID NO: 445 - protein, 9 aa, Homo sapiens
LHITPGTAY

SEQ ID NO: 446 - protein, 9 aa, Homo sapiens
GRIVAFFSF

SEQ ID NO: 447 - protein, 8 aa, Homo sapiens
MQVLVSRI

SEQ ID NO: 448 - protein, 8 aa, Homo sapiens
LSQKGYSW

SEQ ID NO: 449 - protein, 10 aa, Homo sapiens
RAFSDLTSQL

SEQ ID NO: 450 - protein, 9 aa, Homo sapiens
KQTFPFPTI

SEQ ID NO: 451 - protein, 10 aa, Homo sapiens
DYLNEWGSRF

SEQ ID NO: 452 - protein, 9 aa, Homo sapiens
LKVLGVNVM

SEQ ID NO: 453 - protein, 8 aa, Homo sapiens
DVKLEKPK

SEQ ID NO: 454 - protein, 9 aa, Homo sapiens
AQTDPTTGY

SEQ ID NO: 455 - protein, 9 aa, Homo sapiens
AAAANAQVY

SEQ ID NO: 456 - protein, 11 aa, Homo sapiens
IPLERPLGEVY

SEQ ID NO: 457 - protein, 11 aa, Homo sapiens
NAAAAANAQVY

SEQ ID NO: 458 - protein, 8 aa, Homo sapiens
TDTLIHLM

SEQ ID NO: 459 - protein, 9 aa, Homo sapiens
KVAGERYVY

SEQ ID NO: 460 - protein, 11 aa, Homo sapiens
RLSSATANALY

SEQ ID NO: 461 - protein, 9 aa, Homo sapiens
AQRMTTQLL

SEQ ID NO: 462 - protein, 9 aa, Homo sapiens
QRMTTQLLL

SEQ ID NO: 463 - protein, 9 aa, Homo sapiens
VNQSLLDLY

SEQ ID NO: 464 - protein, 8 aa, Homo sapiens
MSALRPLL

SEQ ID NO: 465 - protein, 9 aa, Homo sapiens
DLIESGQLR

SEQ ID NO: 466 - protein, 11 aa, Homo sapiens
DLIESGQLRER

SEQ ID NO: 467 - protein, 9 aa, Homo sapiens
MQMQERDTL

SEQ ID NO: 468 - protein, 8 aa, Homo sapiens
ALAKLLPL

SEQ ID NO: 469 - protein, 9 aa, Homo sapiens
QEQSSVVRA

SEQ ID NO: 470 - protein, 10 aa, Homo sapiens
QGERLLGAAV

SEQ ID NO: 471 - protein, 9 aa, Homo sapiens
AQRLDPVYF

SEQ ID NO: 472 - protein, 8 aa, Homo sapiens
MRLLVAPL

SEQ ID NO: 473 - protein, 10 aa, Homo sapiens
MLNNNALSAL

SEQ ID NO: 474 - protein, 12 aa, Homo sapiens
AADGGLRASVTL

SEQ ID NO: 475 - protein, 10 aa, Homo sapiens
GRDPTSYPSL

SEQ ID NO: 476 - protein, 9 aa, Homo sapiens
ISYPPLHEW

SEQ ID NO: 477 - protein, 9 aa, Homo sapiens
RIQQQTNTY

SEQ ID NO: 478 - protein, 9 aa, Homo sapiens
VVGPKGATI

SEQ ID NO: 479 - protein, 9 aa, Homo sapiens
TEGSHFVEA

SEQ ID NO: 480 - protein, 9 aa, Homo sapiens
GRADIMIDF

SEQ ID NO: 481 - protein, 10 aa, Homo sapiens
GRWEKTDLTY

SEQ ID NO: 482 - protein, 11 aa, Homo sapiens
GRWEKTDLTYR

SEQ ID NO: 483 - protein, 11 aa, Homo sapiens
VRFPVHAALVW

SEQ ID NO: 484 - protein, 8 aa, Homo sapiens
AWLRSAAA

SEQ ID NO: 485 - protein, 9 aa, Homo sapiens
VRFPVHAAL

SEQ ID NO: 486 - protein, 8 aa, Homo sapiens
DRFFWLKV

SEQ ID NO: 487 - protein, 9 aa, Homo sapiens
GMADILVVF

SEQ ID NO: 488 - protein, 9 aa, Homo sapiens
RSFSLGVPR

SEQ ID NO: 489 - protein, 9 aa, Homo sapiens
EVSGLSTER

SEQ ID NO: 490 - protein, 9 aa, Homo sapiens
AEVQKLLGP

SEQ ID NO: 491 - protein, 9 aa, Homo sapiens
EAYSSTSSW

SEQ ID NO: 492 - protein, 10 aa, Homo sapiens
EVTPWISLTL

SEQ ID NO: 493 - protein, 9 aa, Homo sapiens
DTNLEPVTR

SEQ ID NO: 494 - protein, 9 aa, Homo sapiens
ETTASLVSR

SEQ ID NO: 495 - protein, 12 aa, Homo sapiens
EVPSGATTEVSR

SEQ ID NO: 496 - protein, 12 aa, Homo sapiens
EVPTGTTAEVSR

SEQ ID NO: 497 - protein, 11 aa, Homo sapiens
EVSRTEVISSR

SEQ ID NO: 498 - protein, 11 aa, Homo sapiens
EVYPELGTQGR

SEQ ID NO: 499 - protein, 9 aa, Homo sapiens
SSETTKIKR

SEQ ID NO: 500 - protein, 8 aa, Homo sapiens
AHVLHSTL

SEQ ID NO: 501 - protein, 9 aa, Homo sapiens
IQIEPTSSL

SEQ ID NO: 502 - protein, 9 aa, Homo sapiens
SGDQGITSL

SEQ ID NO: 503 - protein, 10 aa, Homo sapiens
TVFDKAFTAA

SEQ ID NO: 504 - protein, 9 aa, Homo sapiens
TVSSVNQGL

SEQ ID NO: 505 - protein, 10 aa, Homo sapiens
YVPTGAITQA

SEQ ID NO: 506 - protein, 10 aa, Homo sapiens
HQFITSTNTF

SEQ ID NO: 507 - protein, 9 aa, Homo sapiens
TSIFSGQSL

SEQ ID NO: 508 - protein, 9 aa, Homo sapiens
TVAKTTTTF

SEQ ID NO: 509 - protein, 9 aa, Homo sapiens
GRGPGGVSW

SEQ ID NO: 510 - protein, 9 aa, Homo sapiens
RRIPTEPTF

SEQ ID NO: 511 - protein, 9 aa, Homo sapiens
SRIPQDVSW

SEQ ID NO: 512 - protein, 9 aa, Homo sapiens
SRSPENPSW

SEQ ID NO: 513 - protein, 9 aa, Homo sapiens
SRTEISSSR

SEQ ID NO: 514 - protein, 9 aa, Homo sapiens
SRTEVASSR

SEQ ID NO: 515 - protein, 9 aa, Homo sapiens
TRIEMESTF

SEQ ID NO: 516 - protein, 9 aa, Homo sapiens
TASTPISTF

SEQ ID NO: 517 - protein, 11 aa, Homo sapiens
TAETILTFHAF

SEQ ID NO: 518 - protein, 9 aa, Homo sapiens
TSDFPTITV

SEQ ID NO: 519 - protein, 10 aa, Homo sapiens
VTSLLTPGMV

SEQ ID NO: 520 - protein, 9 aa, Homo sapiens
THSAMTHGF

SEQ ID NO: 521 - protein, 9 aa, Homo sapiens
THSTASQGF

SEQ ID NO: 522 - protein, 9 aa, Homo sapiens
THSTISQGF

SEQ ID NO: 523 - protein, 12 aa, Homo sapiens
APKGIPVKPTSA

SEQ ID NO: 524 - protein, 9 aa, Homo sapiens
AVSPTVQGL

SEQ ID NO: 525 - protein, 8 aa, Homo sapiens
QRFPHSEM

SEQ ID NO: 526 - protein, 8 aa, Homo sapiens
SVPDILST

SEQ ID NO: 527 - protein, 9 aa, Homo sapiens
QSTPYVNSV

SEQ ID NO: 528 - protein, 9 aa, Homo sapiens
TRTGLFLRF

SEQ ID NO: 529 - protein, 8 aa, Homo sapiens
PFSNPRVL

SEQ ID NO: 530 - protein, 8 aa, Homo sapiens
MLPRAALL

SEQ ID NO: 531 - protein, 9 aa, Homo sapiens
QGAQLRGAL

SEQ ID NO: 532 - protein, 9 aa, Homo sapiens
AISFSYKAW

SEQ ID NO: 533 - protein, 9 aa, Homo sapiens
GQHLHLETF

SEQ ID NO: 534 - protein, 10 aa, Homo sapiens
CRPGALQIEL

SEQ ID NO: 535 - protein, 8 aa, Homo sapiens
IKDVRKIK

SEQ ID NO: 536 - protein, 10 aa, Homo sapiens
VQDQACVAKF

SEQ ID NO: 537 - protein, 10 aa, Homo sapiens
IRRLKELKDQ

SEQ ID NO: 538 - protein, 9 aa, Homo sapiens
QLEKALKEI

SEQ ID NO: 539 - protein, 11 aa, Homo sapiens
IPIPSTGSVEM

SEQ ID NO: 540 - protein, 9 aa, Homo sapiens
AGIPAVALW

SEQ ID NO: 541 - protein, 9 aa, Homo sapiens
RLSPAPLKL

SEQ ID NO: 542 - protein, 10 aa, Homo sapiens
QIIDEEETQF

SEQ ID NO: 543 - protein, 9 aa, Homo sapiens
MRLSPAPLK

SEQ ID NO: 544 - protein, 9 aa, Homo sapiens
LRNPSIQKL

SEQ ID NO: 545 - protein, 8 aa, Homo sapiens
RVGPPLLI

SEQ ID NO: 546 - protein, 9 aa, Homo sapiens
GRAFFAAAF

SEQ ID NO: 547 - protein, 10 aa, Homo sapiens
EVNKPGVYTR

SEQ ID NO: 548 - protein, 10 aa, Homo sapiens
VSEASLVSSI

SEQ ID NO: 549 - protein, 9 aa, Homo sapiens
ARSKLQQGL

SEQ ID NO: 550 - protein, 9 aa, Homo sapiens
RRFKEPWFL

SEQ ID NO: 551 - protein, 10 aa, Homo sapiens
RLHTGEKPYK

SEQ ID NO: 552 - protein, 20 aa, Homo sapiens
GVNAMLRKVAVAAASKPHVE

SEQ ID NO: 553 - protein, 19 aa, Homo sapiens
VNAMLRKVAVAAASKPHVE

SEQ ID NO: 554 - protein, 18 aa, Homo sapiens
GVNAMLRKVAVAAASKPH

SEQ ID NO: 555 - protein, 17 aa, Homo sapiens
VNAMLRKVAVAAASKPH

SEQ ID NO: 556 - protein, 16 aa, Homo sapiens
NAMLRKVAVAAASKPH

SEQ ID NO: 557 - protein, 15 aa, Homo sapiens
AMLRKVAVAAASKPH

SEQ ID NO: 558 - protein, 13 aa, Homo sapiens
LRKVAVAAASKPH

SEQ ID NO: 559 - protein, 12 aa, Homo sapiens
RKVAVAAASKPH

SEQ ID NO: 560 - protein, 20 aa, Homo sapiens
PNFSGNWKIIRSENFEELLK

SEQ ID NO: 561 - protein, 19 aa, Homo sapiens
PNFSGNWKIIRSENFEELL

SEQ ID NO: 562 - protein, 18 aa, Homo sapiens
GNWKIIRSENFEELLKVL

SEQ ID NO: 563 - protein, 18 aa, Homo sapiens
PNFSGNWKIIRSENFEEL

SEQ ID NO: 564 - protein, 17 aa, Homo sapiens
GNWKIIRSENFEELLKV

SEQ ID NO: 565 - protein, 16 aa, Homo sapiens
NWKIIRSENFEELLKV

SEQ ID NO: 566 - protein, 15 aa, Homo sapiens
NWKIIRSENFEELLK

SEQ ID NO: 567 - protein, 14 aa, Homo sapiens
NWKIIRSENFEELL

SEQ ID NO: 568 - protein, 14 aa, Homo sapiens
WKIIRSENFEELLK

SEQ ID NO: 569 - protein, 13 aa, Homo sapiens
WKIIRSENFEELL

SEQ ID NO: 570 - protein, 11 aa, Homo sapiens
GNWKIIRSENF

SEQ ID NO: 571 - protein, 11 aa, Homo sapiens
PNFSGNWKIIR

SEQ ID NO: 572 - protein, 14 aa, Homo sapiens
INFKVGEEFEEQTV

SEQ ID NO: 573 - protein, 14 aa, Homo sapiens
RLLSADTKGWVRLQ

SEQ ID NO: 574 - protein, 18 aa, Homo sapiens
LPDFYNDWMFIAKHLPDL

SEQ ID NO: 575 - protein, 17 aa, Homo sapiens
VGDDHLLLLQGEQLRRT

SEQ ID NO: 576 - protein, 16 aa, Homo sapiens
VGDDHLLLLQGEQLRR

SEQ ID NO: 577 - protein, 15 aa, Homo sapiens
GDDHLLLLQGEQLRR

SEQ ID NO: 578 - protein, 14 aa, Homo sapiens
DDHLLLLQGEQLRR

SEQ ID NO: 579 - protein, 16 aa, Homo sapiens
SGGPLVCDETLQGILS

SEQ ID NO: 580 - protein, 15 aa, Homo sapiens
GGPLVCDETLQGILS

SEQ ID NO: 581 - protein, 14 aa, Homo sapiens
GGPLVCDETLQGIL

SEQ ID NO: 582 - protein, 16 aa, Homo sapiens
GSQPWQVSLFNGLSFH

SEQ ID NO: 583 - protein, 24 aa, Homo sapiens
LTVKLPDGYEFKFPNRLNLEAINY

SEQ ID NO: 584 - protein, 23 aa, Homo sapiens
TVKLPDGYEFKFPNRLNLEAINY

SEQ ID NO: 585 - protein, 19 aa, Homo sapiens
LTVKLPDGYEFKFPNRLNL

SEQ ID NO: 586 - protein, 18 aa, Homo sapiens
TVKLPDGYEFKFPNRLNL

SEQ ID NO: 587 - protein, 23 aa, Homo sapiens
DQANLTVKLPDGYEFKFPNRLNL

SEQ ID NO: 588 - protein, 19 aa, Homo sapiens
VAPDAKSFVLNLGKDSNNL

SEQ ID NO: 589 - protein, 18 aa, Homo sapiens
APDAKSFVLNLGKDSNNL

SEQ ID NO: 590 - protein, 18 aa, Homo sapiens
RVRGEVAPDAKSFVLNLG

SEQ ID NO: 591 - protein, 16 aa, Homo sapiens
VRGEVAPDAKSFVLNL

SEQ ID NO: 592 - protein, 17 aa, Homo sapiens
VRGEVAPDAKSFVLNLG

SEQ ID NO: 593 - protein, 15 aa, Homo sapiens
GEVAPDAKSFVLNLG

SEQ ID NO: 594 - protein, 15 aa, Homo sapiens
VRGEVAPDAKSFVLN

SEQ ID NO: 595 - protein, 14 aa, Homo sapiens
VRGEVAPDAKSFVL

SEQ ID NO: 596 - protein, 15 aa, Homo sapiens
MAADGDFKIKCVAFD

SEQ ID NO: 597 - protein, 19 aa, Homo sapiens
SPDAESLFREALSNKVDEL

SEQ ID NO: 598 - protein, 16 aa, Homo sapiens
AESLFREALSNKVDEL

SEQ ID NO: 599 - protein, 15 aa, Homo sapiens
AESLFREALSNKVDE

SEQ ID NO: 600 - protein, 11 aa, Homo sapiens
FREALSNKVDE

SEQ ID NO: 601 - protein, 15 aa, Homo sapiens
LSNKVDELAHFLLRK

SEQ ID NO: 602 - protein, 13 aa, Homo sapiens
KDPVAWEAGMLMH

SEQ ID NO: 603 - protein, 13 aa, Homo sapiens
KARDETRGLNVPQ

SEQ ID NO: 604 - protein, 17 aa, Homo sapiens
KLITQDLVKLKYLEYRQ

SEQ ID NO: 605 - protein, 25 aa, Homo sapiens
LTVAEVQKLLGPHVEGLKAEERHRP

SEQ ID NO: 606 - protein, 22 aa, Homo sapiens
LTVAEVQKLLGPHVEGLKAEER

SEQ ID NO: 607 - protein, 21 aa, Homo sapiens
LTVAEVQKLLGPHVEGLKAEE

SEQ ID NO: 608 - protein, 20 aa, Homo sapiens
LTVAEVQKLLGPHVEGLKAE

SEQ ID NO: 609 - protein, 19 aa, Homo sapiens
LTVAEVQKLLGPHVEGLKA

SEQ ID NO: 610 - protein, 18 aa, Homo sapiens
LTVAEVQKLLGPHVEGLK

SEQ ID NO: 611 - protein, 17 aa, Homo sapiens
LTVAEVQKLLGPHVEGL

SEQ ID NO: 612 - protein, 17 aa, Homo sapiens
TVAEVQKLLGPHVEGLK

SEQ ID NO: 613 - protein, 16 aa, Homo sapiens
LTVAEVQKLLGPHVEG

SEQ ID NO: 614 - protein, 16 aa, Homo sapiens
TVAEVQKLLGPHVEGL

SEQ ID NO: 615 - protein, 16 aa, Homo sapiens
VAEVQKLLGPHVEGLK

SEQ ID NO: 616 - protein, 15 aa, Homo sapiens
TVAEVQKLLGPHVEG

SEQ ID NO: 617 - protein, 15 aa, Homo sapiens
VAEVQKLLGPHVEGL

SEQ ID NO: 618 - protein, 14 aa, Homo sapiens
VAEVQKLLGPHVEG

SEQ ID NO: 619 - protein, 13 aa, Homo sapiens
VAEVQKLLGPHVE

SEQ ID NO: 620 - protein, 12 aa, Homo sapiens
EVQKLLGPHVEG

SEQ ID NO: 621 - protein, 11 aa, Homo sapiens
LTVAEVQKLLG

SEQ ID NO: 622 - protein, 25 aa, Homo sapiens
MDALRGLLPVLGQPIIRSIPQGIVA

SEQ ID NO: 623 - protein, 23 aa, Homo sapiens
ALRGLLPVLGQPIIRSIPQGIVA

SEQ ID NO: 624 - protein, 22 aa, Homo sapiens
LRGLLPVLGQPIIRSIPQGIVA

SEQ ID NO: 625 - protein, 21 aa, Homo sapiens
DALRGLLPVLGQPIIRSIPQG

SEQ ID NO: 626 - protein, 21 aa, Homo sapiens
RGLLPVLGQPIIRSIPQGIVA

SEQ ID NO: 627 - protein, 20 aa, Homo sapiens
ALRGLLPVLGQPIIRSIPQG

SEQ ID NO: 628 - protein, 20 aa, Homo sapiens
DALRGLLPVLGQPIIRSIPQ

SEQ ID NO: 629 - protein, 20 aa, Homo sapiens
GLLPVLGQPIIRSIPQGIVA

SEQ ID NO: 630 - protein, 19 aa, Homo sapiens
ALRGLLPVLGQPIIRSIPQ

SEQ ID NO: 631 - protein, 19 aa, Homo sapiens
DALRGLLPVLGQPIIRSIP

SEQ ID NO: 632 - protein, 19 aa, Homo sapiens
LLPVLGQPIIRSIPQGIVA

SEQ ID NO: 633 - protein, 18 aa, Homo sapiens
LRGLLPVLGQPIIRSIPQ

SEQ ID NO: 634 - protein, 17 aa, Homo sapiens
DALRGLLPVLGQPIIRS

SEQ ID NO: 635 - protein, 16 aa, Homo sapiens
ALRGLLPVLGQPIIRS

SEQ ID NO: 636 - protein, 16 aa, Homo sapiens
DALRGLLPVLGQPIIR

SEQ ID NO: 637 - protein, 15 aa, Homo sapiens
ALRGLLPVLGQPIIR

SEQ ID NO: 638 - protein, 15 aa, Homo sapiens
LRGLLPVLGQPIIRS

SEQ ID NO: 639 - protein, 14 aa, Homo sapiens
ALRGLLPVLGQPII

SEQ ID NO: 640 - protein, 13 aa, Homo sapiens
ALRGLLPVLGQPI

SEQ ID NO: 641 - protein, 13 aa, Homo sapiens
RGLLPVLGQPIIR

SEQ ID NO: 642 - protein, 12 aa, Homo sapiens
GLLPVLGQPIIR

SEQ ID NO: 643 - protein, 12 aa, Homo sapiens
LRGLLPVLGQPI

SEQ ID NO: 644 - protein, 11 aa, Homo sapiens
RGLLPVLGQPI

SEQ ID NO: 645 - protein, 25 aa, Homo sapiens
RGLLPVLGQPIIRSIPQGIVAAWRQ

SEQ ID NO: 646 - protein, 24 aa, Homo sapiens
GLLPVLGQPIIRSIPQGIVAAWRQ

SEQ ID NO: 647 - protein, 22 aa, Homo sapiens
LPVLGQPIIRSIPQGIVAAWRQ

SEQ ID NO: 648 - protein, 21 aa, Homo sapiens
GLLPVLGQPIIRSIPQGIVAA

SEQ ID NO: 649 - protein, 20 aa, Homo sapiens
LLPVLGQPIIRSIPQGIVAA

SEQ ID NO: 650 - protein, 20 aa, Homo sapiens
LPVLGQPIIRSIPQGIVAAW

SEQ ID NO: 651 - protein, 19 aa, Homo sapiens
LPVLGQPIIRSIPQGIVAA

SEQ ID NO: 652 - protein, 19 aa, Homo sapiens
PVLGQPIIRSIPQGIVAAW

SEQ ID NO: 653 - protein, 18 aa, Homo sapiens
LPVLGQPIIRSIPQGIVA

SEQ ID NO: 654 - protein, 17 aa, Homo sapiens
PVLGQPIIRSIPQGIVA

SEQ ID NO: 655 - protein, 16 aa, Homo sapiens
LGQPIIRSIPQGIVAA

SEQ ID NO: 656 - protein, 16 aa, Homo sapiens
VLGQPIIRSIPQGIVA

SEQ ID NO: 657 - protein, 13 aa, Homo sapiens
QPIIRSIPQGIVA

SEQ ID NO: 658 - protein, 25 aa, Homo sapiens
VSTMDALRGLLPVLGQPIIRSIPQG

SEQ ID NO: 659 - protein, 24 aa, Homo sapiens
VSTMDALRGLLPVLGQPIIRSIPQ

SEQ ID NO: 660 - protein, 20 aa, Homo sapiens
VSTMDALRGLLPVLGQPIIR

SEQ ID NO: 661 - protein, 19 aa, Homo sapiens
LRGLLPVLGQPIIRSIPQG

SEQ ID NO: 662 - protein, 24 aa, Homo sapiens
LRTDAVLPLTVAEVQKLLGPHVEG

SEQ ID NO: 663 - protein, 23 aa, Homo sapiens
RTDAVLPLTVAEVQKLLGPHVEG

SEQ ID NO: 664 - protein, 20 aa, Homo sapiens
AVLPLTVAEVQKLLGPHVEG

SEQ ID NO: 665 - protein, 19 aa, Homo sapiens
VLPLTVAEVQKLLGPHVEG

SEQ ID NO: 666 - protein, 18 aa, Homo sapiens
LPLTVAEVQKLLGPHVEG

SEQ ID NO: 667 - protein, 13 aa, Homo sapiens
TDAVLPLTVAEVQ

SEQ ID NO: 668 - protein, 12 aa, Homo sapiens
AVLPLTVAEVQK

SEQ ID NO: 669 - protein, 24 aa, Homo sapiens
VLPLTVAEVQKLLGPHVEGLKAEE

SEQ ID NO: 670 - protein, 21 aa, Homo sapiens
VLPLTVAEVQKLLGPHVEGLK

SEQ ID NO: 671 - protein, 20 aa, Homo sapiens
LPLTVAEVQKLLGPHVEGLK

SEQ ID NO: 672 - protein, 23 aa, Homo sapiens
LRGLLPVLGQPIIRSIPQGIVAA

SEQ ID NO: 673 - protein, 21 aa, Homo sapiens
IPFTYEQLDVLKHKLDELYPQ

SEQ ID NO: 674 - protein, 17 aa, Homo sapiens
IPFTYEQLDVLKHKLDE

SEQ ID NO: 675 - protein, 16 aa, Homo sapiens
IPFTYEQLDVLKHKLD

SEQ ID NO: 676 - protein, 20 aa, Homo sapiens
VPPSSIWAVRPQDLDTCDPR

SEQ ID NO: 677 - protein, 15 aa, Homo sapiens
IWAVRPQDLDTCDPR

SEQ ID NO: 678 - protein, 13 aa, Homo sapiens
AVRPQDLDTCDPR

SEQ ID NO: 679 - protein, 20 aa, Homo sapiens
WGVRGSLLSEADVRALGGLA

SEQ ID NO: 680 - protein, 19 aa, Homo sapiens
GVRGSLLSEADVRALGGLA

SEQ ID NO: 681 - protein, 19 aa, Homo sapiens
WGVRGSLLSEADVRALGGL

SEQ ID NO: 682 - protein, 18 aa, Homo sapiens
GVRGSLLSEADVRALGGL

SEQ ID NO: 683 - protein, 18 aa, Homo sapiens
VRGSLLSEADVRALGGLA

SEQ ID NO: 684 - protein, 18 aa, Homo sapiens
WGVRGSLLSEADVRALGG

SEQ ID NO: 685 - protein, 17 aa, Homo sapiens
GVRGSLLSEADVRALGG

SEQ ID NO: 686 - protein, 17 aa, Homo sapiens
VRGSLLSEADVRALGGL

SEQ ID NO: 687 - protein, 17 aa, Homo sapiens
WGVRGSLLSEADVRALG

SEQ ID NO: 688 - protein, 16 aa, Homo sapiens
GVRGSLLSEADVRALG

SEQ ID NO: 689 - protein, 16 aa, Homo sapiens
WGVRGSLLSEADVRAL

SEQ ID NO: 690 - protein, 15 aa, Homo sapiens
GSLLSEADVRALGGL

SEQ ID NO: 691 - protein, 15 aa, Homo sapiens
GVRGSLLSEADVRAL

SEQ ID NO: 692 - protein, 15 aa, Homo sapiens
RGSLLSEADVRALGG

SEQ ID NO: 693 - protein, 15 aa, Homo sapiens
WGVRGSLLSEADVRA

SEQ ID NO: 694 - protein, 14 aa, Homo sapiens
GSLLSEADVRALGG

SEQ ID NO: 695 - protein, 14 aa, Homo sapiens
RGSLLSEADVRALG

SEQ ID NO: 696 - protein, 14 aa, Homo sapiens
WGVRGSLLSEADVR

SEQ ID NO: 697 - protein, 13 aa, Homo sapiens
GSLLSEADVRALG

SEQ ID NO: 698 - protein, 13 aa, Homo sapiens
VRGSLLSEADVRA

SEQ ID NO: 699 - protein, 12 aa, Homo sapiens
LLSEADVRALGG

SEQ ID NO: 700 - protein, 12 aa, Homo sapiens
SLLSEADVRALG

SEQ ID NO: 701 - protein, 11 aa, Homo sapiens
GSLLSEADVRA

SEQ ID NO: 702 - protein, 11 aa, Homo sapiens
LLSEADVRALG

SEQ ID NO: 703 - protein, 11 aa, Homo sapiens
LSEADVRALGG

SEQ ID NO: 704 - protein, 10 aa, Homo sapiens
SEADVRALGG

SEQ ID NO: 705 - protein, 9 aa, Homo sapiens
EADVRALGG

SEQ ID NO: 706 - protein, 19 aa, Homo sapiens
LSTERVRELAVALAQKNVK

SEQ ID NO: 707 - protein, 17 aa, Homo sapiens
LSTERVRELAVALAQKN

SEQ ID NO: 708 - protein, 16 aa, Homo sapiens
ERVRELAVALAQKNVK

SEQ ID NO: 709 - protein, 16 aa, Homo sapiens
LSTERVRELAVALAQK

SEQ ID NO: 710 - protein, 15 aa, Homo sapiens
LSTERVRELAVALAQ

SEQ ID NO: 711 - protein, 15 aa, Homo sapiens
STERVRELAVALAQK

SEQ ID NO: 712 - protein, 15 aa, Homo sapiens
TERVRELAVALAQKN

SEQ ID NO: 713 - protein, 14 aa, Homo sapiens
VRELAVALAQKNVK

SEQ ID NO: 714 - protein, 18 aa, Homo sapiens
AIPFTYEQLDVLKHKLDE

SEQ ID NO: 715 - protein, 18 aa, Homo sapiens
GLSTERVRELAVALAQKN

SEQ ID NO: 716 - protein, 16 aa, Homo sapiens
GLSTERVRELAVALAQ

SEQ ID NO: 717 - protein, 18 aa, Homo sapiens
IPQGIVAAWRQRSSRDPS

SEQ ID NO: 718 - protein, 15 aa, Homo sapiens
GIVAAWRQRSSRDPS

SEQ ID NO: 719 - protein, 15 aa, Homo sapiens
IPQGIVAAWRQRSSR

SEQ ID NO: 720 - protein, 17 aa, Homo sapiens
ALGGLACDLPGRFVAES

SEQ ID NO: 721 - protein, 17 aa, Homo sapiens
RELAVALAQKNVKLSTE

SEQ ID NO: 722 - protein, 16 aa, Homo sapiens
LKALLEVNKGHEMSPQ

SEQ ID NO: 723 - protein, 16 aa, Homo sapiens
TFMKLRTDAVLPLTVA

SEQ ID NO: 724 - protein, 15 aa, Homo sapiens
FMKLRTDAVLPLTVA

SEQ ID NO: 725 - protein, 13 aa, Homo sapiens
FMKLRTDAVLPLT

SEQ ID NO: 726 - protein, 12 aa, Homo sapiens
FMKLRTDAVLPL

SEQ ID NO: 727 - protein, 16 aa, Homo sapiens
TLGLGLQGGIPNGYLV

SEQ ID NO: 728 - protein, 15 aa, Homo sapiens
DLPGRFVAESAEVLL

SEQ ID NO: 729 - protein, 14 aa, Homo sapiens
DLPGRFVAESAEVL

SEQ ID NO: 730 - protein, 13 aa, Homo sapiens
LPGRFVAESAEVL

SEQ ID NO: 731 - protein, 11 aa, Homo sapiens
DLPGRFVAESA

SEQ ID NO: 732 - protein, 15 aa, Homo sapiens
ERHRPVRDWILRQRQ

SEQ ID NO: 733 - protein, 15 aa, Homo sapiens
SPRQLLGFPCAEVSG

SEQ ID NO: 734 - protein, 15 aa, Homo sapiens
SRTLAGETGQEAAPL

SEQ ID NO: 735 - protein, 15 aa, Homo sapiens
VTSLETLKALLEVNK

SEQ ID NO: 736 - protein, 14 aa, Homo sapiens
LGLQGGIPNGYLVL

SEQ ID NO: 737 - protein, 12 aa, Homo sapiens
LQGGIPNGYLVL

SEQ ID NO: 738 - protein, 10 aa, Homo sapiens
GGIPNGYLVL

SEQ ID NO: 739 - protein, 14 aa, Homo sapiens
LQGGIPNGYLVLDL

SEQ ID NO: 740 - protein, 13 aa, Homo sapiens
APERQRLLPAALA

SEQ ID NO: 741 - protein, 13 aa, Homo sapiens
FVKIQSFLGGAPT

SEQ ID NO: 742 - protein, 10 aa, Homo sapiens
FVKIQSFLGG

SEQ ID NO: 743 - protein, 9 aa, Homo sapiens
FVKIQSFLG

SEQ ID NO: 744 - protein, 11 aa, Homo sapiens
FLKMSPEDIRK

SEQ ID NO: 745 - protein, 21 aa, Homo sapiens
WELSQLTNSVTELGPYTLDRD

SEQ ID NO: 746 - protein, 20 aa, Homo sapiens
EITITTQTGYSLATSQVTLP

SEQ ID NO: 747 - protein, 19 aa, Homo sapiens
ATTPSWVETHSIVIQGFPH

SEQ ID NO: 748 - protein, 19 aa, Homo sapiens
GIKELGPYTLDRNSLYVNG

SEQ ID NO: 749 - protein, 15 aa, Homo sapiens
GIKELGPYTLDRNSL

SEQ ID NO: 750 - protein, 14 aa, Homo sapiens
GPYTLDRNSLYVNG

SEQ ID NO: 751 - protein, 13 aa, Homo sapiens
GIKELGPYTLDRN

SEQ ID NO: 752 - protein, 13 aa, Homo sapiens
LGPYTLDRNSLYV

SEQ ID NO: 753 - protein, 12 aa, Homo sapiens
LGPYTLDRNSLY

SEQ ID NO: 754 - protein, 11 aa, Homo sapiens
LGPYTLDRNSL

SEQ ID NO: 755 - protein, 17 aa, Homo sapiens
IELGPYLLDRGSLYVNG

SEQ ID NO: 756 - protein, 15 aa, Homo sapiens
LGPYLLDRGSLYVNG

SEQ ID NO: 757 - protein, 14 aa, Homo sapiens
LGPYLLDRGSLYVN

SEQ ID NO: 758 - protein, 13 aa, Homo sapiens
LGPYLLDRGSLYV

SEQ ID NO: 759 - protein, 17 aa, Homo sapiens
EELGPYTLDRNSLYVNG

SEQ ID NO: 760 - protein, 16 aa, Homo sapiens
LKPLFKSTSVGPLYSG

SEQ ID NO: 761 - protein, 15 aa, Homo sapiens
LKPLFKSTSVGPLYS

SEQ ID NO: 762 - protein, 14 aa, Homo sapiens
LKPLFKSTSVGPLY

SEQ ID NO: 763 - protein, 13 aa, Homo sapiens
LKPLFKSTSVGPL

SEQ ID NO: 764 - protein, 16 aa, Homo sapiens
FDKAFTAATTEVSRTE

SEQ ID NO: 765 - protein, 15 aa, Homo sapiens
ELGPYTLDRDSLYVN

SEQ ID NO: 766 - protein, 15 aa, Homo sapiens
GLLKPLFKSTSVGPL

SEQ ID NO: 767 - protein, 14 aa, Homo sapiens
LLKPLFKSTSVGPL

SEQ ID NO: 768 - protein, 15 aa, Homo sapiens
SDPYKATSAVVITST

SEQ ID NO: 769 - protein, 14 aa, Homo sapiens
SDPYKATSAVVITS

SEQ ID NO: 770 - protein, 15 aa, Homo sapiens
SRKFNTMESVLQGLL

SEQ ID NO: 771 - protein, 13 aa, Homo sapiens
SRKFNTMESVLQG

SEQ ID NO: 772 - protein, 14 aa, Homo sapiens
LGFYVLDRDSLFIN

SEQ ID NO: 773 - protein, 9 aa, Homo sapiens
ALYGKLLKL

SEQ ID NO: 774 - protein, 9 aa, Homo sapiens
VYVDDIYVI

SEQ ID NO: 775 - protein, 10 aa, Homo sapiens
ELAGIGILTV

SEQ ID NO: 776 - protein, 9 aa, Homo sapiens
YLLPAIVHI